European Patent Application EP 4 253 566 A1, published October 4, 2023. Title: MARKER OF CALCIUM-OVERLOAD-MEDIATED NEURONAL DEATH AND APPLICATION THEREOF. Applicant: 首都医科大学. The sequence listing filed with the application follows.

SEQUENCE LISTING (33 sequences)

SEQ ID NO: 1 - DNA, 25 bp, synthetic construct
  source 1..25: mol_type = other DNA
taggtgttagtaagggaccacttaa

SEQ ID NO: 2 - DNA, 25 bp, synthetic construct
  source 1..25: mol_type = other DNA
cgtcggatccttgagtgataaagaa

SEQ ID NO: 3 - DNA, 25 bp, synthetic construct
  source 1..25: mol_type = other DNA
gaccgcttgagactgggccacttta

SEQ ID NO: 4 - DNA, 25 bp, synthetic construct
  source 1..25: mol_type = other DNA
gaggaggtttcagtgaagtttacaa

SEQ ID NO: 5 - DNA, 25 bp, synthetic construct
  source 1..25: mol_type = other DNA
cagagcaaagatacgtagctgtgaa

SEQ ID NO: 6 - DNA, 25 bp, synthetic construct
  source 1..25: mol_type = other DNA
catgtagggaataccggattcataa

SEQ ID NO: 7 - DNA, 25 bp, synthetic construct
  source 1..25: mol_type = other DNA
ggaaatgatctggacttctacctga

SEQ ID NO: 8 - DNA, 25 bp, synthetic construct
  source 1..25: mol_type = other DNA
cccggtccattatcatgcagattgt

SEQ ID NO: 9 - DNA, 25 bp, synthetic construct
  source 1..25: mol_type = other DNA
ggtccattatcatgcagattgtgaa

SEQ ID NO: 10 - DNA, 25 bp, synthetic construct
  source 1..25: mol_type = other DNA
tgatgtccagcagctggcctgtgat

SEQ ID NO: 11 - DNA, 25 bp, synthetic construct
  source 1..25: mol_type = other DNA
cctcttctgggaatacagagctaaa

SEQ ID NO: 12 - DNA, 25 bp, synthetic construct
  source 1..25: mol_type = other DNA
taggagcccacagtttacttaggtt

SEQ ID NO: 13 - DNA, 25 bp, synthetic construct
  source 1..25: mol_type = other DNA
ccacagtttacttaggttaacgtta

SEQ ID NO: 14 - DNA, 19 bp, synthetic construct
  source 1..19: mol_type = other DNA
gtcggatccttgagtgata

SEQ ID NO: 15 - DNA, 19 bp, synthetic construct
  source 1..19: mol_type = other DNA
ccattatcatgcagattgt

SEQ ID NO: 16 - DNA, 19 bp, synthetic construct
  source 1..19: mol_type = other DNA
cgacacggagcctcattta

SEQ ID NO: 17 - DNA, 19 bp, synthetic construct
  source 1..19: mol_type = other DNA
cgaagatcatggatgatga

SEQ ID NO: 18 - DNA, 19 bp, synthetic construct
  source 1..19: mol_type = other DNA
ggagctgctattgcatcaa

SEQ ID NO: 19 - DNA, 19 bp, synthetic construct
  source 1..19: mol_type = other DNA
agcagaataccatgaacaa

SEQ ID NO: 20 - DNA, 19 bp, synthetic construct
  source 1..19: mol_type = other DNA
gagctggagagactagaaa

SEQ ID NO: 21 - DNA, 19 bp, synthetic construct
  source 1..19: mol_type = other DNA
ccaacgctaaatgacagat

SEQ ID NO: 22 - DNA, 19 bp, synthetic construct
  source 1..19: mol_type = other DNA
agagcaaagatacgtagct

SEQ ID NO: 23 - DNA, 19 bp, synthetic construct
  source 1..19: mol_type = other DNA
gcaagtacgtggcaatgtt

SEQ ID NO: 24 - DNA, 19 bp, synthetic construct
  source 1..19: mol_type = other DNA
ggttagaagactgcagctt

SEQ ID NO: 25 - DNA, 19 bp, synthetic construct
  source 1..19: mol_type = other DNA
ggaagatggagtgtttcaa

SEQ ID NO: 26 - DNA, 19 bp, synthetic construct
  source 1..19: mol_type = other DNA
gcacatataaacgtgtgca

SEQ ID NO: 27 - DNA, 19 bp, synthetic construct
  source 1..19: mol_type = other DNA
gctggatcatcccagaata

SEQ ID NO: 28 - DNA, 19 bp, synthetic construct
  source 1..19: mol_type = other DNA
gcagattgtgaatgcttta

SEQ ID NO: 29 - DNA, 19 bp, synthetic construct
  source 1..19: mol_type = other DNA
cctcaaaccaggtaatatt

SEQ ID NO: 30 - DNA, 19 bp, synthetic construct
  source 1..19: mol_type = other DNA
gctggtacttattggtatt

SEQ ID NO: 31 - DNA, 19 bp, synthetic construct
  source 1..19: mol_type = other DNA
gccagtagtaacacctgaa

SEQ ID NO: 32 - DNA, 19 bp, synthetic construct
  source 1..19: mol_type = other DNA
gcgtccaataacagttctt

SEQ ID NO: 33 - DNA, 19 bp, synthetic construct
  source 1..19: mol_type = other DNA
gccagtgaaatcactaagt